European Patent Application EP 4 707 396 A1, published March 11, 2026. Title: Method and expression system for producing biologically active molecules. Applicant: Ningaloo Biosystems GmbH. Application EP. The sequence listing filed with the application follows.

SEQUENCE LISTING (10 sequences)

SEQ ID NO: 1 - protein, 755 aa, synthetic construct
PKKKRKVDALDDFDLDMLGSDALDDFDLDMLGSDALDDFDLDMLGSDALDDFDLDMLAAAEFQYLPDTDDRHRIEEKRKRTYETFKSIMKKSPFSGPTDPRPPPRRIAVPSRSSASVPKPAPQPYPFTSSLSTINYDEFPTMVFPSGQISQASALAPAPPQVLPQAPAPAPAPAMVSALAQAPAPVPVLAPGPPQAVAPPAPKPTQAGEGTLSEALLQLQFDDEDLGALLGNSTDPAVFTDLASVDNSEFQQLLNQGIPVAPHTTEPMLMEYPEAITRLVTGAQRPPDPAPAPLGAPGLPNGLLSGDEDFSSIADMDFSALLSQISSGSGSGSRDSREGMFLPKPEAGSAISDVFEGREVCQPKRIRPFHPPGSPWANRPLPASLAPTPTGPVHEPVGSLTPAPVPQPLDPAPAVTPEASHLLEDPDEETSQAVKALREMADTVIPQKEEAAICGQMDLSHPPPRGHLDELTTTLESMTEDLNLDSPLTPELNEILDTFLNDECLLHAMHISTGLSIFDTSLFEFGADDTRVEVQPPAQWVLDLIEASPIASVVSDPRLADNPLIAINQAFTDLTGYSEEECVGRNCRFLAGSGTEPWLTDKIRQGVREHKPVLVEILNYKKDGTPFRNAVLVAPIYDDDDELLYFLGSQVEVDDDQPNMGMARRERAAEMLRTLSPRQLEVTTLVASGLRNKEVAARLGLSEKTVKMHRGLVMEKLNLKTSADLVRIAVEAGIEFSASKRPAATKKAGQAKKKK

SEQ ID NO: 2 - protein, 7 aa, synthetic construct
PKKKRKV

SEQ ID NO: 3 - protein, 50 aa, synthetic construct
DALDDFDLDMLGSDALDDFDLDMLGSDALDDFDLDMLGSDALDDFDLDML

SEQ ID NO: 4 - skipped

SEQ ID NO: 5 - protein, 267 aa, synthetic construct
EFQYLPDTDDRHRIEEKRKRTYETFKSIMKKSPFSGPTDPRPPPRRIAVPSRSSASVPKPAPQPYPFTSSLSTINYDEFPTMVFPSGQISQASALAPAPPQVLPQAPAPAPAPAMVSALAQAPAPVPVLAPGPPQAVAPPAPKPTQAGEGTLSEALLQLQFDDEDLGALLGNSTDPAVFTDLASVDNSEFQQLLNQGIPVAPHTTEPMLMEYPEAITRLVTGAQRPPDPAPAPLGAPGLPNGLLSGDEDFSSIADMDFSALLSQISS

SEQ ID NO: 6 - protein, 6 aa, synthetic construct
GSGSGS

SEQ ID NO: 7 - protein, 190 aa, synthetic construct
RDSREGMFLPKPEAGSAISDVFEGREVCQPKRIRPFHPPGSPWANRPLPASLAPTPTGPVHEPVGSLTPAPVPQPLDPAPAVTPEASHLLEDPDEETSQAVKALREMADTVIPQKEEAAICGQMDLSHPPPRGHLDELTTTLESMTEDLNLDSPLTPELNEILDTFLNDECLLHAMHISTGLSIFDTSLF

SEQ ID NO: 8 - protein, 734 aa, synthetic construct
PKKKRKVDALDDFDLDMLGSDALDDFDLDMLGSDALDDFDLDMLGSDALDDFDLDMLAAAEFQYLPDTDDRHRIEEKRKRTYETFKSIMKKSPFSGPTDPRPPPRRIAVPSRSSASVPKPAPQPYPFTSSLSTINYDEFPTMVFPSGQISQASALAPAPPQVLPQAPAPAPAPAMVSALAQAPAPVPVLAPGPPQAVAPPAPKPTQAGEGTLSEALLQLQFDDEDLGALLGNSTDPAVFTDLASVDNSEFQQLLNQGIPVAPHTTEPMLMEYPEAITRLVTGAQRPPDPAPAPLGAPGLPNGLLSGDEDFSSIADMDFSALLSQISSGSGSGSRDSREGMFLPKPEAGSAISDVFEGREVCQPKRIRPFHPPGSPWANRPLPASLAPTPTGPVHEPVGSLTPAPVPQPLDPAPAVTPEASHLLEDPDEETSQAVKALREMADTVIPQKEEAAICGQMDLSHPPPRGHLDELTTTLESMTEDLNLDSPLTPELNEILDTFLNDECLLHAMHISTGLSIFDTSLFEFGADDTRVEVQPPAQWVLDLIEASPIASVVSDPRLADNPLIAINQAFTDLTGYSEEECVGRNCRFLAGSGTEPWLTDKIRQGVREHKPVLVEILNYKKDGTPFRNAVLVAPIYDDDDELLYFLGSQVEVDDDQPNMGMARRERAAEMLRTLSPRQLEVTTLVASGLRNKEVAARLGLSEKTVKMHRGLVMEKLNLKTSADLVRIAVEAGI

SEQ ID NO: 9 - protein, 5 aa, synthetic construct
EFSAS

SEQ ID NO: 10 - protein, 16 aa, synthetic construct
KRPAATKKAGQAKKKK